European Patent Application EP 4 660 301 A1, published December 10, 2025. Title: Modified polypeptide having protease activity. Applicant: CJ CheilJedang Corporation. The sequence listing filed with the application follows.

SEQUENCE LISTING (18 sequences)

SEQ ID NO: 1 - protein, 380 aa, Alkalihalobacillus clausii
MKKPLGKIVASTALLISVAFSSSIASAAEEAKEKYLIGFNEQEAVSEFVEQVEANDEVAILSEEEEVEIELLHEFETIPVLSVELSPEDVDALELDPAISYIEEDAEVTTMAQSVPWGISRVQAPAAHNRGLTGSGVKVAVLDTGISTHPDLNIRGGASFVPGEPSTQDGNGHGTHVAGTIAALNNSIGVLGVAPSAELYAVKVLGASGSGSVSSIAQGLEWAGNNGMHVANLSLGSPSPSATLEQAVNSATSRGVLVVAASGNSGAGSISYPARYANAMAVGATDQNNNRASFSQYGAGLDIVAPGVNVQSTYPGSTYASLNGTSMATPHVAGAAALVKQKNPSWSNVQIRNHLKNTATSLGSTNLYGSGLVNAEAATR

SEQ ID NO: 2 - protein, 380 aa, synthetic construct
MKKPLGKIVASTALLISVAFSSSIASAAEEAKEKYLIGFNEQEAVSEFVEQVEANDEVAILSEEEEVEIELLHEFETIPVLSVELSPEDVDALELDPAISYIEEDAEVTTMAQSVPWGIARVQAPAAHNRGLTGSGVKVAVLDTGISTHPDLDIRGGASFVPGEPSTQDGNGHGTHVAGTIAALDNSIGVLGVAPSAELYAVKVLGASGSGSVSSIAQGLEWAGNNGMHVANLSLGSPSPSATLEQAVNSATSRGVLVVAASGNSGAGSISYPARYANAMAVGATDQNNNRAPFSQYGAGLDIVAPGVNVQSTYPGSTYASLSGTSMATPHVAGAAALVKQKNPSWSNKQIRNHLKNTATPLGSTNLYGSGLVNAEAATR

SEQ ID NO: 3 - DNA, 1143 bp, Alkalihalobacillus clausii
  source 1..1143: mol_type = genomic DNA
atgaagaaaccgttggggaaaattgtcgcaagcaccgcactactcatttctgttgcttttagttcatcgatcgcatcggctgctgaagaagcaaaagaaaaatatttaattggctttaatgagcaggaagctgtcagtgagtttgtagaacaagtagaggcaaatgacgaggtcgccattctctctgaggaagaggaagtcgaaattgaattgcttcatgaatttgaaacgattcctgttttatccgttgagttaagcccagaagatgtggacgcgcttgaactcgatccagcgatttcttatattgaagaggatgcagaagtaacgacaatggcgcaatcagtgccatggggaattagccgtgtgcaagccccagctgcccataaccgtggattgacaggttctggtgtaaaagttgctgtcctcgatacaggtatttccactcatccagacttaaatattcgtggtggcgctagctttgtaccaggggaaccatccactcaagatgggaatgggcatggcacacatgtggccgggacgattgctgctttaaacaattcgattggcgttcttggcgtagcgccgagcgcggaactatacgctgttaaagtattaggggcgagcggttcaggttcggtcagctcgattgcccaaggattggaatgggcagggaacaatggcatgcacgttgctaatttgagtttaggaagcccttcgccaagtgccacacttgagcaagctgttaatagcgcgacttctagaggcgttcttgttgtagcggcatctgggaattcaggtgcaggctcaatcagctatccggcccgttatgcgaacgcaatggcagtcggagctactgaccaaaacaacaaccgcgccagcttttcacagtatggcgcagggcttgacattgtcgcaccaggtgtaaacgtgcagagcacatacccaggttcaacgtatgccagcttaaacggtacatcgatggctactcctcatgttgcaggtgcagcagcccttgttaaacaaaagaacccatcttggtccaatgtacaaatccgcaatcatctaaagaatacggcaacgagcttaggaagcacgaacttgtatggaagcggacttgtcaatgcagaagcggcaacacgctaa

SEQ ID NO: 4 - DNA, 1143 bp, synthetic construct
  source 1..1143: mol_type = other DNA
atgaagaaaccgttggggaaaattgtcgcaagcaccgcactactcatttctgttgcttttagttcatcgatcgcatcggctgctgaagaagcaaaagaaaaatatttaattggctttaatgagcaggaagctgtcagtgagtttgtagaacaagtagaggcaaatgacgaggtcgccattctctctgaggaagaggaagtcgaaattgaattgcttcatgaatttgaaacgattcctgttttatccgttgagttaagcccagaagatgtggacgcgcttgaactcgatccagcgatttcttatattgaagaggatgcagaagtaacgacaatggcgcaatcagtgccatggggaattgcccgtgtgcaagccccagctgcccataaccgtggattgacaggttctggtgtaaaagttgctgtcctcgatacaggtatttccactcatccagacttagacattcgtggtggcgctagctttgtaccaggggaaccatccactcaagatgggaatgggcatggcacacatgtggccgggacgattgctgctttagacaattcgattggcgttcttggcgtagcgccgagcgcggaactatacgctgttaaagtattaggggcgagcggttcaggttcggtcagctcgattgcccaaggattggaatgggcagggaacaatggcatgcacgttgctaatttgagtttaggaagcccttcgccaagtgccacacttgagcaagctgttaatagcgcgacttctagaggcgttcttgttgtagcggcatctgggaattcaggtgcaggctcaatcagctatccggcccgttatgcgaacgcaatggcagtcggagctactgaccaaaacaacaaccgcgccccattttcacagtatggcgcagggcttgacattgtcgcaccaggtgtaaacgtgcagagcacatacccaggttcaacgtatgccagcttaagcggtacatcgatggctactcctcatgttgcaggtgcagcagcccttgttaaacaaaagaacccatcttggtccaataaacaaatccgcaatcatctaaagaatacggcaacgccattaggaagcacgaacttgtatggaagcggacttgtcaatgcagaagcggcaacacgctaa

SEQ ID NO: 5 - DNA, 30 bp, synthetic construct
  source 1..30: mol_type = other DNA; note = S120A_F
gtgccatggggaattgcccgtgtgcaagcc

SEQ ID NO: 6 - DNA, 17 bp, synthetic construct
  source 1..17: mol_type = other DNA; note = S120A_R
aattccccatggcactg

SEQ ID NO: 7 - DNA, 28 bp, synthetic construct
  source 1..28: mol_type = other DNA; note = N153D_F
catccagacttagacattcgtggtggcg

SEQ ID NO: 8 - DNA, 16 bp, synthetic construct
  source 1..16: mol_type = other DNA; note = N153D_R
cactcatccagactta

SEQ ID NO: 9 - DNA, 33 bp, synthetic construct
  source 1..33: mol_type = other DNA; note = N185D_F
acgattgctgctttagacaattcgattggcgtt

SEQ ID NO: 10 - DNA, 16 bp, synthetic construct
  source 1..16: mol_type = other DNA; note = N185D_R
taaagcagcaatcgtc

SEQ ID NO: 11 - DNA, 29 bp, synthetic construct
  source 1..29: mol_type = other DNA; note = S293P_F
aacaaccgcgccccattttcacagtatgg

SEQ ID NO: 12 - DNA, 16 bp, synthetic construct
  source 1..16: mol_type = other DNA; note = S293P_R
ggcgcggttgttgttt

SEQ ID NO: 13 - DNA, 33 bp, synthetic construct
  source 1..33: mol_type = other DNA; note = N323S_F
acgtatgccagcttaagcggtacatcgatggct

SEQ ID NO: 14 - DNA, 16 bp, synthetic construct
  source 1..16: mol_type = other DNA; note = N323S_R
taagctggcatacgtt

SEQ ID NO: 15 - DNA, 27 bp, synthetic construct
  source 1..27: mol_type = other DNA; note = V349K_F
tcttggtccaataaacaaatccgcaat

SEQ ID NO: 16 - DNA, 16 bp, synthetic construct
  source 1..16: mol_type = other DNA; note = V349K_R
attggaccaagatggg

SEQ ID NO: 17 - DNA, 29 bp, synthetic construct
  source 1..29: mol_type = other DNA; note = S361P_F
aatacggcaacgccattaggaagcacgaa

SEQ ID NO: 18 - DNA, 16 bp, synthetic construct
  source 1..16: mol_type = other DNA; note = S361P_R
cgttgccgtattcttt